European Patent Application EP 4 353 252 A1, published April 17, 2024. Title: ANTIGEN-SPECIFIC T CELLS BY GENE EDITING OF CD3 EPSILON. Applicant: Charité Universitätsmedizin Berlin. The sequence listing filed with the application follows.

SEQUENCE LISTING (58 sequences)

SEQ ID NO: 1 - RNA, 23 nt, synthetic construct
  source 1..23: mol_type = other RNA
ggggcaagatggtgagatatgct

SEQ ID NO: 2 - RNA, 23 nt, synthetic construct
  source 1..23: mol_type = other RNA
tagttggcgtttgggggcaagat

SEQ ID NO: 3 - RNA, 23 nt, synthetic construct
  source 1..23: mol_type = other RNA
ttttctagttggcgtttgggggc

SEQ ID NO: 4 - RNA, 23 nt, synthetic construct
  source 1..23: mol_type = other RNA
tccccagcatataaagtctccat

SEQ ID NO: 5 - RNA, 23 nt, synthetic construct
  source 1..23: mol_type = other RNA
agatccaggatactgagggcatg

SEQ ID NO: 6 - RNA, 20 nt, synthetic construct
  source 1..20: mol_type = other RNA
agggcatgtcaatattactg

SEQ ID NO: 7 - RNA, 20 nt, synthetic construct
  source 1..20: mol_type = other RNA
gatgaggatgataaaaacat

SEQ ID NO: 8 - RNA, 20 nt, synthetic construct
  source 1..20: mol_type = other RNA
gttggcgtttgggggcaaga

SEQ ID NO: 9 - RNA, 20 nt, synthetic construct
  source 1..20: mol_type = other RNA
gagaatcaaaatcggtgaat

SEQ ID NO: 10 - DNA, 1613 bp, synthetic construct
  source 1..1613: mol_type = other DNA
tacccaaccaagagcgtgtttttcttccacagacaccaatgttcaaaatggaggcttgggggcaaaattcttttgctatgtctctagtcgtccaaaaaatggtcctaactttttctgactcctgcttgtcaaaaattgtgggctcatagttaatgctagatgcttccttcctctatttccccccaaatttcctgggaacccctggtcaataccagcagtaagttccactgttctagggtgtagaaatggctgtgacccagcagcaagagggaaggacatcagatgtcatcagtggtcatactgcaacacagccctttttctgtttaggaatgcaggtacccacaacatttactaacactttttttttcttatttattttctagttggcgtttgggggcaagagcagaagctcatcagtgaagaagatctgcaagtgcaactggtgcagtcaggaggaggagttgtgcagccaggaggaagtctgcgggtcagttgcgccgcgtcaggcgttactctctccgattatggaatgcattgggtcagacaggcaccaggcaaaggtctggaatggatggcattcattcgcaatgacgggtcggataagtattacgctgacagcgtaaagggcaggtttacaatctctcgggataatagcaaaaaaactgtcagcctgcagatgagttcactgcgcgccgaggacaccgctgtgtactattgtgctaaaaacggcgagtctgggccattggattattggtactttgatctctgggggcggggaacactggtgactgtgtctggaggtggtggatcaggaggtggaggttccggaggtggaggaagtgacgtcgtgatgactcagtctccctcctctctgagtgccagcgttggggatcgcgttacgatcacctgccaagccagccaggatatcagcaactacttaaattggtatcagcaaaagcctggaaaggctccaaagctgctaatctacgacgcgtccaacctggagaccggtgttccatcacgcttctctggatctgggtctggtaccgattttacattcaccatatcttctttgcaacccgaggacttcgctacctattattgccaacagtatagcagcttccctttaactttcgggggaggcactaaagtggatatcaagcggggaggcggaggtagcggaggcggcggaagcggtggaggtgggtctcaagatggtgagatatgctttctttctttcttttttatgaaatcaccccatcattctttgtagttatgaatggagctttctcttaggcctcccacagaacttccacagaggtcaggaaaaggagtttctgccatctacccctttgactttcctcacaagtctggagatatttctagcccagaagagggaagcaacagaggcaggaaataatgagtcttaaccatacaaaagaaaaattgagacttaaatgaagttgaaagcactaacagttttcatttgtttgcatttcatatttgatgtgagattctgcagaggagacgtagccagaatgcatgcacagggttactctggataagctgctggggcaacatttggatgtgtgttcagaatcacatgtctgaat

SEQ ID NO: 11 - DNA, 400 bp, synthetic construct
  source 1..400: mol_type = other DNA
tacccaaccaagagcgtgtttttcttccacagacaccaatgttcaaaatggaggcttgggggcaaaattcttttgctatgtctctagtcgtccaaaaaatggtcctaactttttctgactcctgcttgtcaaaaattgtgggctcatagttaatgctagatgcttccttcctctatttccccccaaatttcctgggaacccctggtcaataccagcagtaagttccactgttctagggtgtagaaatggctgtgacccagcagcaagagggaaggacatcagatgtcatcagtggtcatactgcaacacagccctttttctgtttaggaatgcaggtacccacaacatttactaacactttttttttcttatttattttctagttggcgtttgggggcaa

SEQ ID NO: 12 - DNA, 30 bp, synthetic construct
  source 1..30: mol_type = other DNA
gagcagaagctcatcagtgaagaagatctg

SEQ ID NO: 13 - DNA, 366 bp, synthetic construct
  source 1..366: mol_type = other DNA
caagtgcaactggtgcagtcaggaggaggagttgtgcagccaggaggaagtctgcgggtcagttgcgccgcgtcaggcgttactctctccgattatggaatgcattgggtcagacaggcaccaggcaaaggtctggaatggatggcattcattcgcaatgacgggtcggataagtattacgctgacagcgtaaagggcaggtttacaatctctcgggataatagcaaaaaaactgtcagcctgcagatgagttcactgcgcgccgaggacaccgctgtgtactattgtgctaaaaacggcgagtctgggccattggattattggtactttgatctctgggggcggggaacactggtgactgtgtct

SEQ ID NO: 14 - DNA, 45 bp, synthetic construct
  source 1..45: mol_type = other DNA
ggaggtggtggatcaggaggtggaggttccggaggtggaggaagt

SEQ ID NO: 15 - DNA, 324 bp, synthetic construct
  source 1..324: mol_type = other DNA
gacgtcgtgatgactcagtctccctcctctctgagtgccagcgttggggatcgcgttacgatcacctgccaagccagccaggatatcagcaactacttaaattggtatcagcaaaagcctggaaaggctccaaagctgctaatctacgacgcgtccaacctggagaccggtgttccatcacgcttctctggatctgggtctggtaccgattttacattcaccatatcttctttgcaacccgaggacttcgctacctattattgccaacagtatagcagcttccctttaactttcgggggaggcactaaagtggatatcaagcgg

SEQ ID NO: 16 - DNA, 45 bp, synthetic construct
  source 1..45: mol_type = other DNA
ggaggcggaggtagcggaggcggcggaagcggtggaggtgggtct

SEQ ID NO: 17 - DNA, 403 bp, synthetic construct
  source 1..403: mol_type = other DNA
caagatggtgagatatgctttctttctttcttttttatgaaatcaccccatcattctttgtagttatgaatggagctttctcttaggcctcccacagaacttccacagaggtcaggaaaaggagtttctgccatctacccctttgactttcctcacaagtctggagatatttctagcccagaagagggaagcaacagaggcaggaaataatgagtcttaaccatacaaaagaaaaattgagacttaaatgaagttgaaagcactaacagttttcatttgtttgcatttcatatttgatgtgagattctgcagaggagacgtagccagaatgcatgcacagggttactctggataagctgctggggcaacatttggatgtgtgttcagaatcacatgtctgaat

SEQ ID NO: 18 - DNA, 1823 bp, synthetic construct
  source 1..1823: mol_type = other DNA
tcttcccagcattgcattctcaactccattttagaaaggttccaaatagggacttctgtgggtttttctttacatccatcttacccttcccaagtccccatgtccctgcgtaaaccctaaagccacctctcaaaaggttctctagttcccttcaaggttctctagttcccttcattccacatatctcctcttccacaccctctagccagtagagctcccttctgacaagcaagtctaagatctagatgacagatgacttcctgcatttgggtggttcttttgtcactaatttgccttttctaaaattgtcctggtttcttctgccaatttcccttctttctccccagcatataaagtctccatctctggaaccacagtaatattgacatgccctcagtatgccaccaacttctctcttttgaagcaggccggagatgtggaagaaaatcctgggcccatgcaatcaggcactcactggcgagtgctgggtctgtgcttgctcagcgtaggagtatggggtcaagagcagaagctcatcagtgaagaagatctgcaagtgcaactggtgcagtcaggaggaggagttgtgcagccaggaggaagtctgcgggtcagttgcgccgcgtcaggcgttactctctccgattatggaatgcattgggtcagacaggcaccaggcaaaggtctggaatggatggcattcattcgcaatgacgggtcggataagtattacgctgacagcgtaaagggcaggtttacaatctctcgggataatagcaaaaaaactgtcagcctgcagatgagttcactgcgcgccgaggacaccgctgtgtactattgtgctaaaaacggcgagtctgggccattggattattggtactttgatctctgggggcggggaacactggtgactgtgtctggaggtggtggatcaggaggtggaggttccggaggtggaggaagtgacgtcgtgatgactcagtctccctcctctctgagtgccagcgttggggatcgcgttacgatcacctgccaagccagccaggatatcagcaactacttaaattggtatcagcaaaagcctggaaaggctccaaagctgctaatctacgacgcgtccaacctggagaccggtgttccatcacgcttctctggatctgggtctggtaccgattttacattcaccatatcttctttgcaacccgaggacttcgctacctattattgccaacagtatagcagcttccctttaactttcgggggaggcactaaagtggatatcaagcggggaggtggtggatcaggaggtggaggttccggaggtggaggaagtgacggtaacgaagagatggggggaatcacccagacaccatacaaagtcagcatcagcggcacaacggtcatcctgacgtgtcctcaataccctggatctgaaatactatggcaacacaatgataaaaacataggcggtgatgaggatgataaaaacataggcagtgatgaggatcacctgtcactgaaggaattttcagaattggagcaaagtggttattatgtctgctaccccagaggaagcaaaccagaagatgcgaacttttatctctacctgagggcaagaggtaatccaggtctccagaacaggtaccaccggctctttagggaggaccattcaaaagggcattctcagtgattttccctaacccagctcacagtgcccaggcgtctttgcgcttcctcccacactcaatcctgggactctctggtaccacacggcatcagtgttttctggaatatagattaaacaccaatatgaggcttctggg

SEQ ID NO: 19 - DNA, 400 bp, synthetic construct
  source 1..400: mol_type = other DNA
tcttcccagcattgcattctcaactccattttagaaaggttccaaatagggacttctgtgggtttttctttacatccatcttacccttcccaagtccccatgtccctgcgtaaaccctaaagccacctctcaaaaggttctctagttcccttcaaggttctctagttcccttcattccacatatctcctcttccacaccctctagccagtagagctcccttctgacaagcaagtctaagatctagatgacagatgacttcctgcatttgggtggttcttttgtcactaatttgccttttctaaaattgtcctggtttcttctgccaatttcccttctttctccccagcatataaagtctccatctctggaaccacagtaatattgacatgccctcagtat

SEQ ID NO: 20 - DNA, 57 bp, synthetic construct
  source 1..57: mol_type = other DNA
gccaccaacttctctcttttgaagcaggccggagatgtggaagaaaatcctgggccc

SEQ ID NO: 21 - DNA, 66 bp, synthetic construct
  source 1..66: mol_type = other DNA
atgcaatcaggcactcactggcgagtgctgggtctgtgcttgctcagcgtaggagtatggggtcaa

SEQ ID NO: 22 - DNA, 30 bp, synthetic construct; identical to SEQ ID NO: 12
  source 1..30: mol_type = other DNA

SEQ ID NO: 23 - DNA, 366 bp, synthetic construct; identical to SEQ ID NO: 13
  source 1..366: mol_type = other DNA

SEQ ID NO: 24 - DNA, 45 bp, synthetic construct; identical to SEQ ID NO: 14
  source 1..45: mol_type = other DNA

SEQ ID NO: 25 - DNA, 324 bp, synthetic construct; identical to SEQ ID NO: 15
  source 1..324: mol_type = other DNA

SEQ ID NO: 26 - DNA, 45 bp, synthetic construct; identical to SEQ ID NO: 14
  source 1..45: mol_type = other DNA

SEQ ID NO: 27 - DNA, 90 bp, synthetic construct
  source 1..90: mol_type = other DNA
gacggtaacgaagagatggggggaatcacccagacaccatacaaagtcagcatcagcggcacaacggtcatcctgacgtgtcctcaatac

SEQ ID NO: 28 - DNA, 400 bp, synthetic construct
  source 1..400: mol_type = other DNA
cctggatctgaaatactatggcaacacaatgataaaaacataggcggtgatgaggatgataaaaacataggcagtgatgaggatcacctgtcactgaaggaattttcagaattggagcaaagtggttattatgtctgctaccccagaggaagcaaaccagaagatgcgaacttttatctctacctgagggcaagaggtaatccaggtctccagaacaggtaccaccggctctttagggaggaccattcaaaagggcattctcagtgattttccctaacccagctcacagtgcccaggcgtctttgcgcttcctcccacactcaatcctgggactctctggtaccacacggcatcagtgttttctggaatatagattaaacaccaatatgaggcttctggg

SEQ ID NO: 29 - DNA, 2823 bp, synthetic construct
  source 1..2823: mol_type = other DNA
cctattaaataaaagaataagcagtattattaagtagccctgcatttcaggtttccttgagtggcaggccaggcctggccgtgaacgttcactgaaatcatggcctcttggccaagattgatagcttgtgcctgtccctgagtcccagtccatcacgagcagctggtttctaagatgctatttcccgtataaagcatgagaccgtgacttgccagccccacagagccccgcccttgtccatcactggcatctggactccagcctgggttggggcaaagagggaaatgagatcatgtcctaaccctgatcctcttgtcccacagatatccagaaccctgaccctgccgtgtaccagctgagagactctaaatccagtgacaagtctgtctgcctattcaccgccaccaacttctctcttttgaagcaggccggagatgtggaagaaaatcctgggcccatggctcttcctgtgactgcccttctgctgcccctggctctcctgctccatgctgcccggccacaagtgcaactggtgcagtcaggaggaggagttgtgcagccaggaggaagtctgcgggtcagttgcgccgcgtcaggcgttactctctccgattatggaatgcattgggtcagacaggcaccaggcaaaggtctggaatggatggcattcattcgcaatgacgggtcggataagtattacgctgacagcgtaaagggcaggtttacaatctctcgggataatagcaaaaaaactgtcagcctgcagatgagttcactgcgcgccgaggacaccgctgtgtactattgtgctaaaaacggcgagtctgggccattggattattggtactttgatctctgggggcggggaacactggtgactgtgtctggaggtggtggatcaggaggtggaggttccggaggtggaggaagtgacgtcgtgatgactcagtctccctcctctctgagtgccagcgttggggatcgcgttacgatcacctgccaagccagccaggatatcagcaactacttaaattggtatcagcaaaagcctggaaaggctccaaagctgctaatctacgacgcgtccaacctggagaccggtgttccatcacgcttctctggatctgggtctggtaccgattttacattcaccatatcttctttgcaacccgaggacttcgctacctattattgccaacagtatagcagcttccctttaactttcgggggaggcactaaagtggatatcaagcgggaaagcaagtatggccccccatgccctccctgccccggacagccgcgggagccccaggtctacaccctcccaccctccagagatgagctgaccaagaaccaggtttcactgacatgcctggtgaagggcttctacccctctgacattgctgtggagtgggagagcaatgggcagccagagaacaactacaagaccacacctcctgtcctggacagcgacggctccttcttcctctacagtaagctcactgtggacaagagccgctggcagcagggcaatgtcttctcctgcagcgtgatgcacgaggccctgcacaatgcctatacccagaagtcactctctctgagccctggaaagaaggatcccaagttttgggtcctcgtggtggtcgggggtgtgctggcctgctacagcttgctggtcacagtggccttcatcatcttctgggtgcgctccaagaggagccggctgcttcacagtgattacatgaacatgacccccaggaggccaggacccaccaggaagcactaccagccctacgctcccccgcgggactttgctgcttaccgcagcagggtcaaattttctagatctgcagatgcgccggcctatcaacaaggccagaaccagctctataacgagctcaatctaggacgaagagaggagtacgatgttttggacaagagacgtggccgggaccctgagatggggggaaagccgagaaggaagaaccctcaggaaggcctgtacaatgaactgcagaaagataagatggcggaggcctacagtgagattgggatgaaaggcgagcgccggaggggcaaggggcacgatggcctttaccagggtctcagtacagccaccaaggacacctacgacgcccttcacatgcaggccctgccccctcgctaataagaattctaactagagctcgctgatcagcctcgactgtgccttctagttgccagccatctgttgtttgcccctcccccgtgccttccttgaccctggaaggtgccactcccactgtcctttcctaataaaatgaggaaattgcatcgcattgtctgagtaggtgtcattctattctggggggtggggtggggcaggacagcaagggggaggattgggaagagaatagcaggcatgctggggagcggccgcgttaaattttgattctcaaacaaatgtgtcacaaagtaaggattctgatgtgtatatcacagacaaaactgtgctagacatgaggtctatggacttcaagagcaacagtgctgtggcctggagcaacaaatctgactttgcatgtgcaaacgccttcaacaacagcattattccagaagacaccttcttccccagcccaggtaagggcagctttggtgccttcgcaggctgtttccttgcttcaggaatggccaggttctgcccagagctctggtcaatgatgtctaaaactcctctgattggtggtctcggccttatccattgccaccaaaaccctctttttactaagaaacagtgagccttgttctggcagtccagagaatgacacgggaaaaaagcagatg

SEQ ID NO: 30 - DNA, 400 bp, synthetic construct
  source 1..400: mol_type = other DNA
cctattaaataaaagaataagcagtattattaagtagccctgcatttcaggtttccttgagtggcaggccaggcctggccgtgaacgttcactgaaatcatggcctcttggccaagattgatagcttgtgcctgtccctgagtcccagtccatcacgagcagctggtttctaagatgctatttcccgtataaagcatgagaccgtgacttgccagccccacagagccccgcccttgtccatcactggcatctggactccagcctgggttggggcaaagagggaaatgagatcatgtcctaaccctgatcctcttgtcccacagatatccagaaccctgaccctgccgtgtaccagctgagagactctaaatccagtgacaagtctgtctgcctattcacc

SEQ ID NO: 31 - DNA, 57 bp, synthetic construct; identical to SEQ ID NO: 20
  source 1..57: mol_type = other DNA

SEQ ID NO: 32 - DNA, 63 bp, synthetic construct
  source 1..63: mol_type = other DNA
atggctcttcctgtgactgcccttctgctgcccctggctctcctgctccatgctgcccggcca

SEQ ID NO: 33 - DNA, 366 bp, synthetic construct; identical to SEQ ID NO: 13
  source 1..366: mol_type = other DNA

SEQ ID NO: 34 - DNA, 45 bp, synthetic construct; identical to SEQ ID NO: 14
  source 1..45: mol_type = other DNA

SEQ ID NO: 35 - DNA, 324 bp, synthetic construct; identical to SEQ ID NO: 15
  source 1..324: mol_type = other DNA

SEQ ID NO: 36 - DNA, 36 bp, synthetic construct
  source 1..36: mol_type = other DNA
gaaagcaagtatggccccccatgccctccctgcccc

SEQ ID NO: 37 - DNA, 321 bp, synthetic construct
  source 1..321: mol_type = other DNA
ggacagccgcgggagccccaggtctacaccctcccaccctccagagatgagctgaccaagaaccaggtttcactgacatgcctggtgaagggcttctacccctctgacattgctgtggagtgggagagcaatgggcagccagagaacaactacaagaccacacctcctgtcctggacagcgacggctccttcttcctctacagtaagctcactgtggacaagagccgctggcagcagggcaatgtcttctcctgcagcgtgatgcacgaggccctgcacaatgcctatacccagaagtcactctctctgagccctggaaag

SEQ ID NO: 38 - DNA, 93 bp, synthetic construct
  source 1..93: mol_type = other DNA
aaggatcccaagttttgggtcctcgtggtggtcgggggtgtgctggcctgctacagcttgctggtcacagtggccttcatcatcttctgggtg

SEQ ID NO: 39 - DNA, 123 bp, synthetic construct
  source 1..123: mol_type = other DNA
cgctccaagaggagccggctgcttcacagtgattacatgaacatgacccccaggaggccaggacccaccaggaagcactaccagccctacgctcccccgcgggactttgctgcttaccgcagc

SEQ ID NO: 40 - DNA, 339 bp, synthetic construct
  source 1..339: mol_type = other DNA
agggtcaaattttctagatctgcagatgcgccggcctatcaacaaggccagaaccagctctataacgagctcaatctaggacgaagagaggagtacgatgttttggacaagagacgtggccgggaccctgagatggggggaaagccgagaaggaagaaccctcaggaaggcctgtacaatgaactgcagaaagataagatggcggaggcctacagtgagattgggatgaaaggcgagcgccggaggggcaaggggcacgatggcctttaccagggtctcagtacagccaccaaggacacctacgacgcccttcacatgcaggccctgccccctcgctaa

SEQ ID NO: 41 - DNA, 257 bp, synthetic construct
  source 1..257: mol_type = other DNA
taagaattctaactagagctcgctgatcagcctcgactgtgccttctagttgccagccatctgttgtttgcccctcccccgtgccttccttgaccctggaaggtgccactcccactgtcctttcctaataaaatgaggaaattgcatcgcattgtctgagtaggtgtcattctattctggggggtggggtggggcaggacagcaagggggaggattgggaagagaatagcaggcatgctggggagcggccgcgttaa

SEQ ID NO: 42 - DNA, 399 bp, synthetic construct
  source 1..399: mol_type = other DNA
attttgattctcaaacaaatgtgtcacaaagtaaggattctgatgtgtatatcacagacaaaactgtgctagacatgaggtctatggacttcaagagcaacagtgctgtggcctggagcaacaaatctgactttgcatgtgcaaacgccttcaacaacagcattattccagaagacaccttcttccccagcccaggtaagggcagctttggtgccttcgcaggctgtttccttgcttcaggaatggccaggttctgcccagagctctggtcaatgatgtctaaaactcctctgattggtggtctcggccttatccattgccaccaaaaccctctttttactaagaaacagtgagccttgttctggcagtccagagaatgacacgggaaaaaagcagatg

SEQ ID NO: 43 - RNA, 25 nt, synthetic construct
  source 1..25: mol_type = other RNA
tcttcccagcattgcattctcaact

SEQ ID NO: 44 - RNA, 29 nt, synthetic construct
  source 1..29: mol_type = other RNA
cccagaagcctcatattggtgtttaatct

SEQ ID NO: 45 - RNA, 25 nt, synthetic construct
  source 1..25: mol_type = other RNA
tacccaaccaagagcgtgtttttct

SEQ ID NO: 46 - RNA, 30 nt, synthetic construct
  source 1..30: mol_type = other RNA
attcagacatgtgattctgaacacacatcc

SEQ ID NO: 47 - protein, 242 aa, synthetic construct
QVQLVQSGGGVVQPGGSLRVSCAASGVTLSDYGMHWVRQAPGKGLEWMAFIRNDGSDKYYADSVKGRFTISRDNSKKTVSLQMSSLRAEDTAVYYCAKNGESGPLDYWYFDLWGRGTLVTVSGGGGSGGGGSGGGGSDVVMTQSPSSLSASVGDRVTITCQASQDISNYLNWYQQKPGKAPKLLIYDASNLETGVPSRFSGSGSGTDFTFTISSLQPEDFATYYCQQYSSFPLTFGGGTKVD

SEQ ID NO: 48 - protein, 122 aa, synthetic construct
QVQLVQSGGGVVQPGGSLRVSCAASGVTLSDYGMHWVRQAPGKGLEWMAFIRNDGSDKYYADSVKGRFTISRDNSKKTVSLQMSSLRAEDTAVYYCAKNGESGPLDYWYFDLWGRGTLVTVS

SEQ ID NO: 49 - protein, 15 aa, synthetic construct
GGGGSGGGGSGGGGS

SEQ ID NO: 50 - protein, 105 aa, synthetic construct
DVVMTQSPSSLSASVGDRVTITCQASQDISNYLNWYQQKPGKAPKLLIYDASNLETGVPSRFSGSGSGTDFTFTISSLQPEDFATYYCQQYSSFPLTFGGGTKVD

SEQ ID NO: 51 - protein, 7 aa, synthetic construct
GVTLSDY

SEQ ID NO: 52 - protein, 6 aa, synthetic construct
RNDGSD

SEQ ID NO: 53 - protein, 14 aa, synthetic construct
NGESGPLDYWYFDL

SEQ ID NO: 54 - protein, 11 aa, synthetic construct
QASQDISNYLN

SEQ ID NO: 55 - protein, 7 aa, synthetic construct
DASNLET

SEQ ID NO: 56 - protein, 9 aa, synthetic construct
QQYSSFPLT

SEQ ID NO: 57 - DNA, 43 bp, synthetic construct
  source 1..43: mol_type = other DNA
cctattaaataaaagaataagcagtattattaagtagccctgc

SEQ ID NO: 58 - DNA, 26 bp, synthetic construct
  source 1..26: mol_type = other DNA
catctgcttttttcccgtgtcattct